European Patent Specification EP 3 639 833 B1, published August 9, 2023. Title: An agent for preventing or treating adipose-related disorders and/or inflammation. Applicant: Biofermin Pharmaceutical Co., Ltd Yokohama City University. The sequence listing filed with the application follows.

SEQUENCE LISTING (12 sequences)

SEQ ID NO: 1 - DNA, 23 bp, Artificial
  Probe
cccgccgatgtcgctatccagct

SEQ ID NO: 2 - DNA, 20 bp, Artificial
  Primer
gaccgatggattcccgttcg

SEQ ID NO: 3 - DNA, 20 bp, Artificial
  Primer
ggacattaggcgcaggaagg

SEQ ID NO: 4 - DNA, 25 bp, Artificial
  Probe
cccagagtggagaagcccagccagt

SEQ ID NO: 5 - DNA, 20 bp, Artificial
  Primer
acccttcagcgttcagcctc

SEQ ID NO: 6 - DNA, 20 bp, Artificial
  Primer
cacacatagctggagcagcg

SEQ ID NO: 7 - DNA, 26 bp, Artificial
  Probe
aggggccaccacgctcttctgtctac

SEQ ID NO: 8 - DNA, 22 bp, Artificial
  Primer
gcctatgtctcagcctcttctc

SEQ ID NO: 9 - DNA, 23 bp, Artificial
  Primer
aggccatttgggaacttctcatc

SEQ ID NO: 10 - DNA, 30 bp, Artificial
  Probe
acaatcagaattgccattgcacaactcttt

SEQ ID NO: 11 - DNA, 20 bp, Artificial
  Primer
gttctctgggaaatcgtgga

SEQ ID NO: 12 - DNA, 20 bp, Artificial
  Primer
ttctgcaagtgcatcatcgt